European Patent Application EP 4 628 099 A2, published October 8, 2025. Title: ENGINEERED EXTRACELLULAR VESICLES AND USES THEREOF. Applicant: LONZA SALES AG. Application EP. The sequence listing filed with the application follows.

SEQUENCE LISTING (425 sequences)

SEQ ID NO: 1 - protein, 332 aa, synthetic construct
  REGION 1..332: note = MARCKS protein
MGAQFSKTAAKGEAAAERPGEAAVASSPSKANGQENGHVKVNGDASPAAAESGAKEELQANGSAPAADKEEPAAAGSGAASPSAAEKGEPAAAAAPEAGASPVEKEAPAEGEAAEPGSPTAAEGEAASAASSTSSPKAEDGATPSPSNETPKKKKKRFSFKKSFKLSGFSFKKNKKEAGEGGEAEAPAAEGGKDEAAGGAAAAAAEAGAASGEQAAAPGEEAAAGEEGAAGGDPQEAKPQEAAVAPEKPPASDETKAAEEPSKVEEKKAEEAGASAAACEAPSAAGPGAPPEQEAAPAEEPAAAAASSACAAPSQEAQPECSPEAPPAEAAE

SEQ ID NO: 2 - protein, 195 aa, synthetic construct
  REGION 1..195: note = MARCKSL1 protein
MGSQSSKAPRGDVTAEEAAGASPAKANGQENGHVKSNGDLSPKGEGESPPVNGTDEAAGATGDAIEPAPPSQGAEAKGEVPPKETPKKKKKFSFKKPFKLSGLSFKRNRKEGGGDSSASSPTEEEQEQGEIGACSDEGTAQEGKAAATPESQEPQAKGAEASAASEEEAGPQATEPSTPSGPESGPTPASAEQNE

SEQ ID NO: 3 - protein, 227 aa, synthetic construct
  REGION 1..227: note = BASP1 protein
MGGKLSKKKKGYNVNDEKAKEKDKKAEGAATEEEGTPKESEPQAAAEPAEAKEGKEKPDQDAEGKAEEKEGEKDAAAAKEEAPKAEPEKTEGAAEAKAEPPKAPEQEQAAPGPAAGGEAPKAAEAAAAPAESAAPAAGEEPSKEEGEPKKTEAPAAPAAQETKSDGAPASDSKPGSSEAAPSSKETPAATEAPSSTPKAQGPAASAEEPKPVEAPAANSDQTVTVKE

SEQ ID NO: 4 - protein, 30 aa, synthetic construct
  REGION 1..30: note = BASP1 fragment
MGGKLSKKKKGYNVNDEKAKEKDKKAEGAA

SEQ ID NO: 5 - protein, 27 aa, synthetic construct
  REGION 1..27: note = fusion protein
MGGKLSKKKKGYNVNDEKAKEKDKKAE

SEQ ID NO: 6 - protein, 24 aa, synthetic construct
  REGION 1..24: note = fusion protein
MGGKLSKKKKGYNVNDEKAKEKDK

SEQ ID NO: 7 - protein, 21 aa, synthetic construct
  REGION 1..21: note = fusion protein
MGGKLSKKKKGYNVNDEKAKE

SEQ ID NO: 8 - protein, 18 aa, synthetic construct
  REGION 1..18: note = fusion protein
MGGKLSKKKKGYNVNDEK

SEQ ID NO: 9 - protein, 15 aa, synthetic construct
  REGION 1..15: note = fusion protein
MGGKLSKKKKGYNVN

SEQ ID NO: 10 - protein, 12 aa, synthetic construct
  REGION 1..12: note = fusion protein
MGGKLSKKKKGY

SEQ ID NO: 11 - protein, 11 aa, synthetic construct
  REGION 1..11: note = fusion protein
MGGKLSKKKKG

SEQ ID NO: 12 - protein, 10 aa, synthetic construct
  REGION 1..10: note = fusion protein
MGGKLSKKKK

SEQ ID NO: 13 - protein, 9 aa, synthetic construct
  REGION 1..9: note = fusion protein
MGGKLSKKK

SEQ ID NO: 14 - protein, 8 aa, synthetic construct
  REGION 1..8: note = fusion protein
MGGKLSKK

SEQ ID NO: 15 - protein, 7 aa, synthetic construct
  REGION 1..7: note = fusion protein
MGGKLSK

SEQ ID NO: 16 - protein, 8 aa, synthetic construct
  REGION 1..8: note = fusion protein
MGGKLAKK

SEQ ID NO: 17 - protein, 8 aa, synthetic construct
  REGION 1..8: note = fusion protein
MGGKFSKK

SEQ ID NO: 18 - protein, 8 aa, synthetic construct
  REGION 1..8: note = fusion protein
MGGKFAKK

SEQ ID NO: 19 - protein, 8 aa, synthetic construct
  REGION 1..8: note = fusion protein
MGGKSSKK

SEQ ID NO: 20 - protein, 8 aa, synthetic construct
  REGION 1..8: note = fusion protein
MGGKSAKK

SEQ ID NO: 21 - protein, 8 aa, synthetic construct
  REGION 1..8: note = fusion protein
MGGKQSKK

SEQ ID NO: 22 - protein, 8 aa, synthetic construct
  REGION 1..8: note = fusion protein
MGGKQAKK

SEQ ID NO: 23 - protein, 8 aa, synthetic construct
  REGION 1..8: note = fusion protein
MGGQLSKK

SEQ ID NO: 24 - protein, 8 aa, synthetic construct
  REGION 1..8: note = fusion protein
MGGQLAKK

SEQ ID NO: 25 - protein, 8 aa, synthetic construct
  REGION 1..8: note = fusion protein
MGGQFSKK

SEQ ID NO: 26 - protein, 8 aa, synthetic construct
  REGION 1..8: note = fusion protein
MGGQFAKK

SEQ ID NO: 27 - protein, 8 aa, synthetic construct
  REGION 1..8: note = fusion protein
MGGQSSKK

SEQ ID NO: 28 - protein, 8 aa, synthetic construct
  REGION 1..8: note = fusion protein
MGGQSAKK

SEQ ID NO: 29 - protein, 8 aa, synthetic construct
  REGION 1..8: note = fusion protein
MGGQQSKK

SEQ ID NO: 30 - protein, 8 aa, synthetic construct
  REGION 1..8: note = fusion protein
MGGQQAKK

SEQ ID NO: 31 - protein, 8 aa, synthetic construct
  REGION 1..8: note = fusion protein
MGAKLSKK

SEQ ID NO: 32 - protein, 8 aa, synthetic construct
  REGION 1..8: note = fusion protein
MGAKLAKK

SEQ ID NO: 33 - protein, 8 aa, synthetic construct
  REGION 1..8: note = fusion protein
MGAKFSKK

SEQ ID NO: 34 - protein, 8 aa, synthetic construct
  REGION 1..8: note = fusion protein
MGAKFAKK

SEQ ID NO: 35 - protein, 8 aa, synthetic construct
  REGION 1..8: note = fusion protein
MGAKSSKK

SEQ ID NO: 36 - protein, 8 aa, synthetic construct
  REGION 1..8: note = fusion protein
MGAKSAKK

SEQ ID NO: 37 - protein, 8 aa, synthetic construct
  REGION 1..8: note = fusion protein
MGAKQSKK

SEQ ID NO: 38 - protein, 8 aa, synthetic construct
  REGION 1..8: note = fusion protein
MGAKQAKK

SEQ ID NO: 39 - protein, 8 aa, synthetic construct
  REGION 1..8: note = fusion protein
MGAQLSKK

SEQ ID NO: 40 - protein, 8 aa, synthetic construct
  REGION 1..8: note = fusion protein
MGAQLAKK

SEQ ID NO: 41 - protein, 8 aa, synthetic construct
  REGION 1..8: note = fusion protein
MGAQFSKK

SEQ ID NO: 42 - protein, 8 aa, synthetic construct
  REGION 1..8: note = fusion protein
MGAQFAKK

SEQ ID NO: 43 - protein, 8 aa, synthetic construct
  REGION 1..8: note = fusion protein
MGAQSSKK

SEQ ID NO: 44 - protein, 8 aa, synthetic construct
  REGION 1..8: note = fusion protein
MGAQSAKK

SEQ ID NO: 45 - protein, 8 aa, synthetic construct
  REGION 1..8: note = fusion protein
MGAQQSKK

SEQ ID NO: 46 - protein, 8 aa, synthetic construct
  REGION 1..8: note = fusion protein
MGAQQAKK

SEQ ID NO: 47 - protein, 8 aa, synthetic construct
  REGION 1..8: note = fusion protein
MGSKLSKK

SEQ ID NO: 48 - protein, 8 aa, synthetic construct
  REGION 1..8: note = fusion protein
MGSKLAKK

SEQ ID NO: 49 - protein, 8 aa, synthetic construct
  REGION 1..8: note = fusion protein
MGSKFSKK

SEQ ID NO: 50 - protein, 8 aa, synthetic construct
  REGION 1..8: note = fusion protein
MGSKFAKK

SEQ ID NO: 51 - protein, 8 aa, synthetic construct
  REGION 1..8: note = fusion protein
MGSKSSKK

SEQ ID NO: 52 - protein, 8 aa, synthetic construct
  REGION 1..8: note = fusion protein
MGSKSAKK

SEQ ID NO: 53 - protein, 8 aa, synthetic construct
  REGION 1..8: note = fusion protein
MGSKQSKK

SEQ ID NO: 54 - protein, 8 aa, synthetic construct
  REGION 1..8: note = fusion protein
MGSKQAKK

SEQ ID NO: 55 - protein, 8 aa, synthetic construct
  REGION 1..8: note = fusion protein
MGSQLSKK

SEQ ID NO: 56 - protein, 8 aa, synthetic construct
  REGION 1..8: note = fusion protein
MGSQLAKK

SEQ ID NO: 57 - protein, 8 aa, synthetic construct
  REGION 1..8: note = fusion protein
MGSQFSKK

SEQ ID NO: 58 - protein, 8 aa, synthetic construct
  REGION 1..8: note = fusion protein
MGSQFAKK

SEQ ID NO: 59 - protein, 8 aa, synthetic construct
  REGION 1..8: note = fusion protein
MGSQSSKK

SEQ ID NO: 60 - protein, 8 aa, synthetic construct
  REGION 1..8: note = fusion protein
MGSQSAKK

SEQ ID NO: 61 - protein, 8 aa, synthetic construct
  REGION 1..8: note = fusion protein
MGSQQSKK

SEQ ID NO: 62 - protein, 8 aa, synthetic construct
  REGION 1..8: note = fusion protein
MGSQQAKK

SEQ ID NO: 63 - protein, 7 aa, synthetic construct
  REGION 1..7: note = fusion protein
MGGKLAK

SEQ ID NO: 64 - protein, 7 aa, synthetic construct
  REGION 1..7: note = fusion protein
MGGKFSK

SEQ ID NO: 65 - protein, 7 aa, synthetic construct
  REGION 1..7: note = fusion protein
MGGKFAK

SEQ ID NO: 66 - protein, 7 aa, synthetic construct
  REGION 1..7: note = fusion protein
MGGKSSK

SEQ ID NO: 67 - protein, 7 aa, synthetic construct
  REGION 1..7: note = fusion protein
MGGKSAK

SEQ ID NO: 68 - protein, 7 aa, synthetic construct
  REGION 1..7: note = fusion protein
MGGKQSK

SEQ ID NO: 69 - protein, 7 aa, synthetic construct
  REGION 1..7: note = fusion protein
MGGKQAK

SEQ ID NO: 70 - protein, 7 aa, synthetic construct
  REGION 1..7: note = fusion protein
MGGQLSK

SEQ ID NO: 71 - protein, 7 aa, synthetic construct
  REGION 1..7: note = fusion protein
MGGQLAK

SEQ ID NO: 72 - protein, 7 aa, synthetic construct
  REGION 1..7: note = fusion protein
MGGQFSK

SEQ ID NO: 73 - protein, 7 aa, synthetic construct
  REGION 1..7: note = fusion protein
MGGQFAK

SEQ ID NO: 74 - protein, 7 aa, synthetic construct
  REGION 1..7: note = fusion protein
MGGQSSK

SEQ ID NO: 75 - protein, 7 aa, synthetic construct
  REGION 1..7: note = fusion protein
MGGQSAK

SEQ ID NO: 76 - protein, 7 aa, synthetic construct
  REGION 1..7: note = fusion protein
MGGQQSK

SEQ ID NO: 77 - protein, 7 aa, synthetic construct
  REGION 1..7: note = fusion protein
MGGQQAK

SEQ ID NO: 78 - protein, 7 aa, synthetic construct
  REGION 1..7: note = fusion protein
MGAKLSK

SEQ ID NO: 79 - protein, 7 aa, synthetic construct
  REGION 1..7: note = fusion protein
MGAKLAK

SEQ ID NO: 80 - protein, 7 aa, synthetic construct
  REGION 1..7: note = fusion protein
MGAKFSK

SEQ ID NO: 81 - protein, 7 aa, synthetic construct
  REGION 1..7: note = fusion protein
MGAKFAK

SEQ ID NO: 82 - protein, 7 aa, synthetic construct
  REGION 1..7: note = fusion protein
MGAKSSK

SEQ ID NO: 83 - protein, 7 aa, synthetic construct
  REGION 1..7: note = fusion protein
MGAKSAK

SEQ ID NO: 84 - protein, 7 aa, synthetic construct
  REGION 1..7: note = fusion protein
MGAKQSK

SEQ ID NO: 85 - protein, 7 aa, synthetic construct
  REGION 1..7: note = fusion protein
MGAKQAK

SEQ ID NO: 86 - protein, 7 aa, synthetic construct
  REGION 1..7: note = fusion protein
MGAQLSK

SEQ ID NO: 87 - protein, 7 aa, synthetic construct
  REGION 1..7: note = fusion protein
MGAQLAK

SEQ ID NO: 88 - protein, 7 aa, synthetic construct
  REGION 1..7: note = fusion protein
MGAQFSK

SEQ ID NO: 89 - protein, 7 aa, synthetic construct
  REGION 1..7: note = fusion protein
MGAQFAK

SEQ ID NO: 90 - protein, 7 aa, synthetic construct
  REGION 1..7: note = fusion protein
MGAQSSK

SEQ ID NO: 91 - protein, 7 aa, synthetic construct
  REGION 1..7: note = fusion protein
MGAQSAK

SEQ ID NO: 92 - protein, 7 aa, synthetic construct
  REGION 1..7: note = fusion protein
MGAQQSK

SEQ ID NO: 93 - protein, 7 aa, synthetic construct
  REGION 1..7: note = fusion protein
MGAQQAK

SEQ ID NO: 94 - protein, 7 aa, synthetic construct
  REGION 1..7: note = fusion protein
MGSKLSK

SEQ ID NO: 95 - protein, 7 aa, synthetic construct
  REGION 1..7: note = fusion protein
MGSKLAK

SEQ ID NO: 96 - protein, 7 aa, synthetic construct
  REGION 1..7: note = fusion protein
MGSKFSK

SEQ ID NO: 97 - protein, 7 aa, synthetic construct
  REGION 1..7: note = fusion protein
MGSKFAK

SEQ ID NO: 98 - protein, 7 aa, synthetic construct
  REGION 1..7: note = fusion protein
MGSKSSK

SEQ ID NO: 99 - protein, 7 aa, synthetic construct
  REGION 1..7: note = fusion protein
MGSKSAK

SEQ ID NO: 100 - protein, 7 aa, synthetic construct
  REGION 1..7: note = fusion protein
MGSKQSK

SEQ ID NO: 101 - protein, 7 aa, synthetic construct
  REGION 1..7: note = fusion protein
MGSKQAK

SEQ ID NO: 102 - protein, 7 aa, synthetic construct
  REGION 1..7: note = fusion protein
MGSQLSK

SEQ ID NO: 103 - protein, 7 aa, synthetic construct
  REGION 1..7: note = fusion protein
MGSQLAK

SEQ ID NO: 104 - protein, 7 aa, synthetic construct
  REGION 1..7: note = fusion protein
MGSQFSK

SEQ ID NO: 105 - protein, 7 aa, synthetic construct
  REGION 1..7: note = fusion protein
MGSQFAK

SEQ ID NO: 106 - protein, 7 aa, synthetic construct
  REGION 1..7: note = fusion protein
MGSQSSK

SEQ ID NO: 107 - protein, 7 aa, synthetic construct
  REGION 1..7: note = fusion protein
MGSQSAK

SEQ ID NO: 108 - protein, 7 aa, synthetic construct
  REGION 1..7: note = fusion protein
MGSQQSK

SEQ ID NO: 109 - protein, 7 aa, synthetic construct
  REGION 1..7: note = fusion protein
MGSQQAK

SEQ ID NO: 110 - protein, 9 aa, synthetic construct
  REGION 1..9: note = scaffold protein
MGAKLSKKK

SEQ ID NO: 111 - protein, 167 aa, synthetic construct
  REGION 1..167: note = scaffold protein
MGGKLSKKKKGYNVNDEKAKEKDKKAEGAASGGSGGSDYKDDDDKGGGSGMASNFTQFVLVDNGGTGDVTVAPSNFANGIAEWISSNSRSQAYKVTCSVRQSSAQNRKYTIKVEVPKGAWRSYLNMELTIPIFATNSDCELIVKAMQGLLKDGNPIPSAIAANSGIY

SEQ ID NO: 112 - protein, 167 aa, synthetic construct
  REGION 1..167: note = scaffold protein
MGGKLSKKKKGYNVNDEKAKEKDKKAEGAASGGSGGSDYKDDDDKGGGSGMASNFTQFVLVDNGGTGDVTVAPSNFANGIAEWISSNSRSQAYKVTCSVRQSSAQKRKYTIKVEVPKGAWRSYLNMELTIPIFATNSDCELIVKAMQGLLKDGNPIPSAIAANSGIY

SEQ ID NO: 113 - protein, 296 aa, synthetic construct
  REGION 1..296: note = scaffold protein
MGGKLSKKKKGYNVNDEKAKEKDKKAEGAASGGSGGSDYKDDDDKGGGSGMASNFTQFVLVDNGGTGDVTVAPSNFANGIAEWISSNSRSQAYKVTCSVRQSSAQNRKYTIKVEVPKGAWRSYLNMELTIPIFATNSDCELIVKAMQGLLKDGNPIPSAIAANSGIYGSGGSGGSGGSGMASNFTQFVLVDNGGTGDVTVAPSNFANGIAEWISSNSRSQAYKVTCSVRQSSAQNRKYTIKVEVPKGAWRSYLNMELTIPIFATNSDCELIVKAMQGLLKDGNPIPSAIAANSGIY

SEQ ID NO: 114 - protein, 296 aa, synthetic construct
  REGION 1..296: note = scaffold protein
MGGKLSKKKKGYNVNDEKAKEKDKKAEGAASGGSGGSDYKDDDDKGGGSGMASNFTQFVLVDNGGTGDVTVAPSNFANGIAEWISSNSRSQAYKVTCSVRQSSAQKRKYTIKVEVPKGAWRSYLNMELTIPIFATNSDCELIVKAMQGLLKDGNPIPSAIAANSGIYGSGGSGGSGGSGMASNFTQFVLVDNGGTGDVTVAPSNFANGIAEWISSNSRSQAYKVTCSVRQSSAQKRKYTIKVEVPKGAWRSYLNMELTIPIFATNSDCELIVKAMQGLLKDGNPIPSAIAANSGIY

SEQ ID NO: 115 - RNA, 680 nt, synthetic construct
  misc_feature 1..680: note = scaffold protein
  source 1..680: mol_type = other RNA
atgaagcccaccgagaacaacgaagacttcaacatcgtggccgtggccagcaacttcgcgaccacggatctcgatgctgaccgcgggaagttgcccggcaagaagctgccgctggaggtgctcaaagagttggaagccaatgcccggaaagctggctgcaccaggggctgtctgatctgcctgtcccacatcaagtgcacgcccaagatgaagaagttcatcccaggacgctgccacacctacgaaggcgacaaagagtccgcacagggcggcataggcgaggcgatcgtcgacattcctgagattcctgggttcaaggacttggagcccttggagcagttcatcgcacaggtcgatctgtgtgtggactgcacaactggctgcctcaaagggcttgccaacgtgcagtgttctgacctgctcaagaagtggctgccgcaacgctgtgcgacctttgccagcaagatccagggccaggtggacaagatcaagggggccggtggtgactaaggatccatcgataagcttcatcgaaacatgaggatcacccatatctgcagtcgacatcgaaacatgaggatcacccatgtctgcagtcgacatcgaaacatgaggatcacccatgtctgcagtcgacatcgaaacatgaggatcacccatgtctgcagtcgacatcgaaa

SEQ ID NO: 116 - protein, 9 aa, synthetic construct
  REGION 1..9: note = scaffold peptide
  SITE 3: note = misc_feature - Xaa can be any naturally occurring amino acid
MGXKLSKKK

SEQ ID NO: 117 - protein, 9 aa, synthetic construct
  REGION 1..9: note = scaffold peptide
  SITE 3: note = misc_feature - Xaa can be any naturally occurring amino acid
MGXKLSKKK

SEQ ID NO: 118 - protein, 8 aa, synthetic construct
  REGION 1..8: note = scaffold protein
  SITE 3: note = MISC_FEATURE - Xaa = G, A, S
  REGION 4: note = MISC_FEATURE - Xaa = K, Q
  SITE 4: note = misc_feature - Xaa can be any naturally occurring amino acid
  SITE 5: note = MISC_FEATURE - Xaa = L, F, S, Q
  SITE 6: note = MISC_FEATURE - Xaa = S, A
MGXXXXKK

SEQ ID NO: 119 - DNA, 20 bp, synthetic construct
  misc_feature 1..20: note = scaffold protein
  source 1..20: mol_type = other DNA
tggaggtgctcaaagagttg

SEQ ID NO: 120 - DNA, 17 bp, synthetic construct
  misc_feature 1..17: note = scaffold protein
  source 1..17: mol_type = other DNA
ttgggcgtgcacttgat

SEQ ID NO: 121 - DNA, 13 bp, synthetic construct
  misc_feature 1..13: note = scaffold protein
  source 1..13: mol_type = other DNA
gggcattggcttc

SEQ ID NO: 122 - protein, 60 aa, synthetic construct
  REGION 1..60: note = scaffold protein
MGGKLSKKKKGYNVNDEKAKEKDKKAEGAASAGGGGSDYKDDDDKGGGGSVSKGEELFTG

SEQ ID NO: 123 - protein, 60 aa, synthetic construct
  REGION 1..60: note = scaffold protein
MAGKLSKKKKGYNVNDEKAKEKDKKAEGAASAGGGGSDYKDDDDKGGGGSVSKGEELFTG

SEQ ID NO: 124 - protein, 60 aa, synthetic construct
  REGION 1..60: note = scaffold protein
MGAKLSKKKKGYNVNDEKAKEKDKKAEGAASAGGGGSDYKDDDDKGGGGSVSKGEELFTG

SEQ ID NO: 125 - protein, 60 aa, synthetic construct
  REGION 1..60: note = scaffold protein
MAAKLSKKKKGYNVNDEKAKEKDKKAEGAASAGGGGSDYKDDDDKGGGGSVSKGEELFTG

SEQ ID NO: 126 - protein, 57 aa, synthetic construct
  REGION 1..57: note = scaffold protein
MGGKLSKKKKGYNVNDEKAKEKDKKAESAGGGGSDYKDDDDKGGGGSVSKGEELFTG

SEQ ID NO: 127 - protein, 54 aa, synthetic construct
  REGION 1..54: note = scaffold protein
MGGKLSKKKKGYNVNDEKAKEKDKSAGGGGSDYKDDDDKGGGGSVSKGEELFTG

SEQ ID NO: 128 - protein, 51 aa, synthetic construct
  REGION 1..51: note = scaffold protein
MGGKLSKKKKGYNVNDEKAKESAGGGGSDYKDDDDKGGGGSVSKGEELFTG

SEQ ID NO: 129 - protein, 48 aa, synthetic construct
  REGION 1..48: note = scaffold protein
MGGKLSKKKKGYNVNDEKSAGGGGSDYKDDDDKGGGGSVSKGEELFTG

SEQ ID NO: 130 - protein, 45 aa, synthetic construct
  REGION 1..45: note = scaffold protein
MGGKLSKKKKGYNVNSAGGGGSDYKDDDDKGGGGSVSKGEELFTG

SEQ ID NO: 131 - protein, 42 aa, synthetic construct
  REGION 1..42: note = scaffold protein
MGGKLSKKKKGYSAGGGGSDYKDDDDKGGGGSVSKGEELFTG

SEQ ID NO: 132 - protein, 39 aa, synthetic construct
  REGION 1..39: note = scaffold protein
MGGKLSKKKSAGGGGSDYKDDDDKGGGGSVSKGEELFTG

SEQ ID NO: 133 - protein, 36 aa, synthetic construct
  REGION 1..36: note = scaffold protein
MGGKLSSAGGGGSDYKDDDDKGGGGSVSKGEELFTG

SEQ ID NO: 134 - protein, 33 aa, synthetic construct
  REGION 1..33: note = scaffold protein
MGGSAGGGGSDYKDDDDKGGGGSVSKGEELFTG

SEQ ID NO: 135 - protein, 54 aa, synthetic construct
  REGION 1..54: note = scaffold protein
MGGKLSKKKKGYNVNDEKAKEKDKKAEGAASAGGGGSDYKDDDDKGGGGSVSKG

SEQ ID NO: 136 - protein, 36 aa, synthetic construct
  REGION 1..36: note = scaffold protein
MGGKLSKKKKGYSAGGGGSDYKDDDDKGGGGSVSKG

SEQ ID NO: 137 - protein, 35 aa, synthetic construct
  REGION 1..35: note = scaffold protein
MGGKLSKKKKGSAGGGGSDYKDDDDKGGGGSVSKG

SEQ ID NO: 138 - protein, 34 aa, synthetic construct
  REGION 1..34: note = scaffold protein
MGGKLSKKKKSAGGGGSDYKDDDDKGGGGSVSKG

SEQ ID NO: 139 - protein, 33 aa, synthetic construct
  REGION 1..33: note = scaffold protein
MGGKLSKKKSAGGGGSDYKDDDDKGGGGSVSKG

SEQ ID NO: 140 - protein, 32 aa, synthetic construct
  REGION 1..32: note = scaffold protein
MGGKLSKKSAGGGGSDYKDDDDKGGGGSVSKG

SEQ ID NO: 141 - protein, 31 aa, synthetic construct
  REGION 1..31: note = scaffold protein
MGGKLSKSAGGGGSDYKDDDDKGGGGSVSKG

SEQ ID NO: 142 - protein, 30 aa, synthetic construct
  REGION 1..30: note = scaffold protein
MGGKLSSAGGGGSDYKDDDDKGGGGSVSKG

SEQ ID NO: 143 - protein, 30 aa, synthetic construct
  REGION 1..30: note = scaffold protein
MGGKLDKKKKGYNVNDEKAKEKDKKAEGAA

SEQ ID NO: 144 - protein, 30 aa, synthetic construct
  REGION 1..30: note = scaffold protein
MGGKLAKKKKGYNVNDEKAKEKDKKAEGAA

SEQ ID NO: 145 - protein, 30 aa, synthetic construct
  REGION 1..30: note = scaffold protein
MGGKQSKKKKGYNVNDEKAKEKDKKAEGAA

SEQ ID NO: 146 - protein, 30 aa, synthetic construct
  REGION 1..30: note = scaffold protein
MGAKKKKKRFSFKKSFKLSGFSFKKNKKEA

SEQ ID NO: 147 - protein, 30 aa, synthetic construct
  REGION 1..30: note = scaffold protein
MAAKKKKKRFSFKKSFKLSGFSFKKNKKEA

SEQ ID NO: 148 - protein, 30 aa, synthetic construct
  REGION 1..30: note = scaffold protein
MGAKKSKKRFSFKKSFKLSGFSFKKNKKEA

SEQ ID NO: 149 - protein, 30 aa, synthetic construct
  REGION 1..30: note = scaffold protein
MGAKKAKKRFSFKKPFKLSGFSFKKNKKEA

SEQ ID NO: 150 - protein, 153 aa, synthetic construct
  REGION 1..153: note = scaffold protein
MGGKLSKKKKSAGGSGGSTSGSGDYKDDDDKGSGFEMDQVQLVESGGALVQPGGSLRLSCAASGFPVNRYSMRWYRQAPGKEREWVAGMSSAGDRSSYEDSVKGRFTISRDDARNTVYLQMNSLKPEDTAVYYCNVNVGFEYWGQGTQVTVSS

SEQ ID NO: 151 - protein, 4 aa, synthetic construct
  REGION 1..4: note = effector domain
KKKK

SEQ ID NO: 152 - protein, 5 aa, synthetic construct
  REGION 1..5: note = effector domain
KKKKK

SEQ ID NO: 153 - protein, 4 aa, synthetic construct
  REGION 1..4: note = effector domain
RRRR

SEQ ID NO: 154 - protein, 5 aa, synthetic construct
  REGION 1..5: note = effector domain
RRRRR

SEQ ID NO: 155-156 - skipped (2 entries)

SEQ ID NO: 157 - protein, 7 aa, synthetic construct
  REGION 1..7: note = scaffold protein
GGKLSKK

SEQ ID NO: 158 - protein, 7 aa, synthetic construct
  REGION 1..7: note = scaffold protein
GAKLSKK

SEQ ID NO: 159 - protein, 7 aa, synthetic construct
  REGION 1..7: note = scaffold protein
GGKQSKK

SEQ ID NO: 160 - protein, 7 aa, synthetic construct
  REGION 1..7: note = scaffold protein
GGKLAKK

SEQ ID NO: 161 - protein, 8 aa, synthetic construct
  REGION 1..8: note = scaffold protein
GGKLSKKK

SEQ ID NO: 162 - protein, 8 aa, synthetic construct
  REGION 1..8: note = scaffold protein
GGKLSKKS

SEQ ID NO: 163 - protein, 8 aa, synthetic construct
  REGION 1..8: note = scaffold protein
GAKLSKKK

SEQ ID NO: 164 - protein, 8 aa, synthetic construct
  REGION 1..8: note = scaffold protein
GAKLSKKS

SEQ ID NO: 165 - protein, 8 aa, synthetic construct
  REGION 1..8: note = scaffold protein
GGKQSKKK

SEQ ID NO: 166 - protein, 8 aa, synthetic construct
  REGION 1..8: note = scaffold protein
GGKQSKKS

SEQ ID NO: 167 - protein, 8 aa, synthetic construct
  REGION 1..8: note = scaffold protein
GGKLAKKK

SEQ ID NO: 168 - protein, 8 aa, synthetic construct
  REGION 1..8: note = scaffold protein
GGKLAKKS

SEQ ID NO: 169 - protein, 14 aa, synthetic construct
  REGION 1..14: note = scaffold protein
GGKLSKKKKGYNVN

SEQ ID NO: 170 - protein, 14 aa, synthetic construct
  REGION 1..14: note = scaffold protein
GAKLSKKKKGYNVN

SEQ ID NO: 171 - protein, 14 aa, synthetic construct
  REGION 1..14: note = scaffold protein
GGKQSKKKKGYNVN

SEQ ID NO: 172 - protein, 14 aa, synthetic construct
  REGION 1..14: note = scaffold protein
GGKLAKKKKGYNVN

SEQ ID NO: 173 - protein, 14 aa, synthetic construct
  REGION 1..14: note = scaffold protein
GGKLSKKKKGYSGG

SEQ ID NO: 174 - protein, 14 aa, synthetic construct
  REGION 1..14: note = scaffold protein
GGKLSKKKKGSGGS

SEQ ID NO: 175 - protein, 14 aa, synthetic construct
  REGION 1..14: note = scaffold protein
GGKLSKKKKSGGSG

SEQ ID NO: 176 - protein, 14 aa, synthetic construct
  REGION 1..14: note = scaffold protein
GGKLSKKKSGGSGG

SEQ ID NO: 177 - protein, 14 aa, synthetic construct
  REGION 1..14: note = scaffold protein
GGKLSKKSGGSGGS

SEQ ID NO: 178 - protein, 14 aa, synthetic construct
  REGION 1..14: note = scaffold protein
GGKLSKSGGSGGSV

SEQ ID NO: 179 - protein, 14 aa, synthetic construct
  REGION 1..14: note = scaffold protein
GAKKSKKRFSFKKS

SEQ ID NO: 180 - protein, 8 aa, synthetic construct
  REGION 1..8: note = scaffold protein
  SITE 4: note = MISC_FEATURE - Xaa= K, Q
  SITE 5: note = MISC_FEATURE - Xaa= L, F, S, Q
  SITE 6: note = MISC_FEATURE - Xaa= S, A
MGGXXXKK

SEQ ID NO: 181 - protein, 8 aa, synthetic construct
  REGION 1..8: note = scaffold protein
  SITE 4: note = MISC_FEATURE - Xaa= K, Q
  SITE 5: note = MISC_FEATURE - Xaa= L, F, S, Q
  SITE 6: note = MISC_FEATURE - Xaa= S, A
MGAXXXKK

SEQ ID NO: 182 - protein, 8 aa, synthetic construct
  REGION 1..8: note = scaffold protein
  SITE 4: note = MISC_FEATURE - Xaa = K, Q
  SITE 5: note = MISC_FEATURE - Xaa = L, F, S, Q
  SITE 6: note = MISC_FEATURE - Xaa = S, A
MGSXXXKK

SEQ ID NO: 183 - protein, 8 aa, synthetic construct
  REGION 1..8: note = scaffold protein
  SITE 3: note = MISC_FEATURE - Xaa = G, A, S
  SITE 5: note = MISC_FEATURE - Xaa = L, F, S, Q
  SITE 6: note = MISC_FEATURE - Xaa = S, A
MGXKXXKK

SEQ ID NO: 184 - protein, 8 aa, synthetic construct
  REGION 1..8: note = scaffold protein
  SITE 3: note = MISC_FEATURE - Xaa= G, A, S
  SITE 5: note = MISC_FEATURE - Xaa= L, F, S, Q
  SITE 6: note = MISC_FEATURE - Xaa= S, A
MGXQXXKK

SEQ ID NO: 185 - protein, 8 aa, synthetic construct
  REGION 1..8: note = scaffold protein
  SITE 3: note = MISC_FEATURE - Xaa = G, A, S
  SITE 4: note = MISC_FEATURE - Xaa = K, Q
  SITE 6: note = MISC_FEATURE - Xaa = S, A
MGXXLXKK

SEQ ID NO: 186 - protein, 8 aa, synthetic construct
  REGION 1..8: note = scaffold protein
  SITE 3: note = MISC_FEATURE - Xaa = G, A, S
  SITE 4: note = MISC_FEATURE - Xaa = K, Q
  SITE 6: note = MISC_FEATURE - Xaa = S, A
MGXXFXKK

SEQ ID NO: 187 - protein, 8 aa, synthetic construct
  REGION 1..8: note = scaffold protein
  SITE 3: note = MISC_FEATURE - Xaa = G, A, S
  SITE 4: note = MISC_FEATURE - Xaa = K, Q
  SITE 6: note = MISC_FEATURE - Xaa = S, A
MGXXSXKK

SEQ ID NO: 188 - protein, 8 aa, synthetic construct
  REGION 1..8: note = scaffold protein
  SITE 3: note = MISC_FEATURE - Xaa = G, A, S
  SITE 4: note = MISC_FEATURE - Xaa = K, Q
  SITE 6: note = MISC_FEATURE - Xaa = S, A
MGXXQXKK

SEQ ID NO: 189 - protein, 8 aa, synthetic construct
  REGION 1..8: note = scaffold protein
  SITE 3: note = MISC_FEATURE - Xaa= G, A, S
  SITE 4: note = MISC_FEATURE - Xaa= K, Q
  SITE 5: note = MISC_FEATURE - Xaa= L, F, S, Q
MGXXXSKK

SEQ ID NO: 190 - protein, 8 aa, synthetic construct
  REGION 1..8: note = scaffold protein
  SITE 3: note = MISC_FEATURE - Xaa = G, A, S
  SITE 4: note = MISC_FEATURE - Xaa = K, Q
  SITE 5: note = MISC_FEATURE - Xaa = L, F, S, Q
MGXXXAKK

SEQ ID NO: 191 - protein, 7 aa, synthetic construct
  REGION 1..7: note = scaffold protein
  SITE 3: note = MISC_FEATURE - Xaa = K, Q
  SITE 4: note = MISC_FEATURE - Xaa = L, F, S, Q
  SITE 5: note = MISC_FEATURE - Xaa = S, A
GGXXXKK

SEQ ID NO: 192 - protein, 7 aa, synthetic construct
  REGION 1..7: note = scaffold protein
  SITE 3: note = MISC_FEATURE - Xaa = K, Q
  SITE 4: note = MISC_FEATURE - Xaa = L, F, S, Q
  SITE 5: note = MISC_FEATURE - Xaa = S, A
GAXXXKK

SEQ ID NO: 193 - protein, 7 aa, synthetic construct
  REGION 1..7: note = scaffold protein
  SITE 3: note = MISC_FEATURE - Xaa = K, Q
  SITE 4: note = MISC_FEATURE - Xaa = L, F, S, Q
  SITE 5: note = MISC_FEATURE - Xaa = S, A
GSXXXKK

SEQ ID NO: 194 - protein, 7 aa, synthetic construct
  REGION 1..7: note = scaffold protein
  SITE 2: note = MISC_FEATURE - Xaa = G, A, S
  SITE 4: note = MISC_FEATURE - Xaa = L, F, S, Q
  SITE 5: note = MISC_FEATURE - Xaa = S, A
GXKXXKK

SEQ ID NO: 195 - protein, 7 aa, synthetic construct
  REGION 1..7: note = scaffold protein
  SITE 2: note = MISC_FEATURE - Xaa = G, A, S
  SITE 4: note = MISC_FEATURE - Xaa = L, F, S, Q
  SITE 5: note = MISC_FEATURE - Xaa = S, A
GXQXXKK

SEQ ID NO: 196 - protein, 7 aa, synthetic construct
  REGION 1..7: note = scaffold protein
  SITE 2: note = MISC_FEATURE - Xaa= G, A, S
  SITE 3: note = MISC_FEATURE - Xaa= K, Q
  SITE 5: note = MISC_FEATURE - Xaa= S, A
GXXLXKK

SEQ ID NO: 197 - protein, 7 aa, synthetic construct
  REGION 1..7: note = scaffold protein
  SITE 2: note = MISC_FEATURE - Xaa = G, A, S
  SITE 3: note = MISC_FEATURE - Xaa = K, Q
  SITE 5: note = MISC_FEATURE - Xaa = S, A
GXXFXKK

SEQ ID NO: 198 - protein, 7 aa, synthetic construct
  REGION 1..7: note = scaffold protein
  SITE 2: note = MISC_FEATURE - Xaa = G, A, S
  SITE 3: note = MISC_FEATURE - Xaa = K, Q
  SITE 5: note = MISC_FEATURE - Xaa = S, A
GXXSXKK

SEQ ID NO: 199 - protein, 7 aa, synthetic construct
  REGION 1..7: note = scaffold protein
  SITE 2: note = MISC_FEATURE - Xaa = G, A, S
  SITE 3: note = MISC_FEATURE - Xaa = K, Q
  SITE 5: note = MISC_FEATURE - Xaa = S, A
GXXQXKK

SEQ ID NO: 200 - protein, 7 aa, synthetic construct
  REGION 1..7: note = scaffold protein
  SITE 2: note = MISC_FEATURE - Xaa = G, A, S
  SITE 3: note = MISC_FEATURE - Xaa = K, Q
  SITE 4: note = MISC_FEATURE - Xaa = L, F, S, Q
GXXXSKK

SEQ ID NO: 201 - protein, 7 aa, synthetic construct
  REGION 1..7: note = scaffold protein
  SITE 2: note = MISC_FEATURE - Xaa = G, A, S
  SITE 3: note = MISC_FEATURE - Xaa = K, Q
  SITE 4: note = MISC_FEATURE - Xaa = L, F, S, Q
GXXXAKK

SEQ ID NO: 202 - skipped

SEQ ID NO: 203 - protein, 6 aa, synthetic construct
  REGION 1..6: note = N-terminus domain
GGKLSK

SEQ ID NO: 204 - protein, 6 aa, synthetic construct
  REGION 1..6: note = N-terminus domain
GAKLSK

SEQ ID NO: 205 - protein, 6 aa, synthetic construct
  REGION 1..6: note = N-terminus domain
GGKQSK

SEQ ID NO: 206 - protein, 6 aa, synthetic construct
  REGION 1..6: note = N-terminus domain
GGKLAK

SEQ ID NO: 207 - protein, 4 aa, synthetic construct
  REGION 1..4: note = N-terminus domain
KKKG

SEQ ID NO: 208 - protein, 5 aa, synthetic construct
  REGION 1..5: note = N-terminus domain
KKKGY

SEQ ID NO: 209 - protein, 6 aa, synthetic construct
  REGION 1..6: note = N-terminus domain
KKKGYN

SEQ ID NO: 210 - protein, 7 aa, synthetic construct
  REGION 1..7: note = N-terminus domain
KKKGYNV

SEQ ID NO: 211 - protein, 8 aa, synthetic construct
  REGION 1..8: note = N-terminus domain
KKKGYNVN

SEQ ID NO: 212 - protein, 6 aa, synthetic construct
  REGION 1..6: note = N-terminus domain
KKKGYS

SEQ ID NO: 213 - protein, 6 aa, synthetic construct
  REGION 1..6: note = N-terminus domain
KKKGYG

SEQ ID NO: 214 - protein, 7 aa, synthetic construct
  REGION 1..7: note = N-terminus domain
KKKGYGG

SEQ ID NO: 215 - protein, 5 aa, synthetic construct
  REGION 1..5: note = N-terminus domain
KKKGS

SEQ ID NO: 216 - protein, 6 aa, synthetic construct
  REGION 1..6: note = N-terminus domain
KKKGSG

SEQ ID NO: 217 - protein, 6 aa, synthetic construct
  REGION 1..6: note = N-terminus domain
KKKGSG

SEQ ID NO: 218 - protein, 7 aa, synthetic construct
  REGION 1..7: note = N-terminus domain
KKKGSGS

SEQ ID NO: 219 - protein, 4 aa, synthetic construct
  REGION 1..4: note = N-terminus domain
KKKS

SEQ ID NO: 220 - protein, 5 aa, synthetic construct
  REGION 1..5: note = N-terminus domain
KKKSG

SEQ ID NO: 221 - protein, 6 aa, synthetic construct
  REGION 1..6: note = N-terminus domain
KKKSGG

SEQ ID NO: 222 - protein, 7 aa, synthetic construct
  REGION 1..7: note = N-terminus domain
KKKSGGS

SEQ ID NO: 223 - protein, 8 aa, synthetic construct
  REGION 1..8: note = N-terminus domain
KKKSGGSG

SEQ ID NO: 224 - protein, 8 aa, synthetic construct
  REGION 1..8: note = N-terminus domain
KKSGGSGG

SEQ ID NO: 225 - protein, 10 aa, synthetic construct
  REGION 1..10: note = N-terminus domain
KKKSGGSGGS

SEQ ID NO: 226 - protein, 8 aa, synthetic construct
  REGION 1..8: note = N-terminus domain
KRFSFKKS

SEQ ID NO: 227 - protein, 29 aa, synthetic construct
  REGION 1..29: note = Scaffold Protein
GGKLSKKKKGYNVNDEKAKEKDKKAEGAA

SEQ ID NO: 228 - protein, 28 aa, synthetic construct
  REGION 1..28: note = Scaffold Protein
GGKLSKKKKGYNVNDEKAKEKDKKAEGA

SEQ ID NO: 229 - protein, 27 aa, synthetic construct
  REGION 1..27: note = Scaffold Protein
GGKLSKKKKGYNVNDEKAKEKDKKAEG

SEQ ID NO: 230 - protein, 26 aa, synthetic construct
  REGION 1..26: note = Scaffold Protein
GGKLSKKKKGYNVNDEKAKEKDKKAE

SEQ ID NO: 231 - protein, 25 aa, synthetic construct
  REGION 1..25: note = Scaffold Protein
GGKLSKKKKGYNVNDEKAKEKDKKA

SEQ ID NO: 232 - protein, 24 aa, synthetic construct
  REGION 1..24: note = Scaffold Protein
GGKLSKKKKGYNVNDEKAKEKDKK

SEQ ID NO: 233 - protein, 23 aa, synthetic construct
  REGION 1..23: note = Scaffold Protein
GGKLSKKKKGYNVNDEKAKEKDK

SEQ ID NO: 234 - protein, 22 aa, synthetic construct
  REGION 1..22: note = Scaffold Protein
GGKLSKKKKGYNVNDEKAKEKD

SEQ ID NO: 235 - protein, 21 aa, synthetic construct
  REGION 1..21: note = Scaffold Protein
GGKLSKKKKGYNVNDEKAKEK

SEQ ID NO: 236 - protein, 20 aa, synthetic construct
  REGION 1..20: note = Scaffold Protein
GGKLSKKKKGYNVNDEKAKE

SEQ ID NO: 237 - protein, 19 aa, synthetic construct
  REGION 1..19: note = Scaffold Protein
GGKLSKKKKGYNVNDEKAK

SEQ ID NO: 238 - protein, 18 aa, synthetic construct
  REGION 1..18: note = Scaffold Protein
GGKLSKKKKGYNVNDEKA

SEQ ID NO: 239 - protein, 17 aa, synthetic construct
  REGION 1..17: note = Scaffold Protein
GGKLSKKKKGYNVNDEK

SEQ ID NO: 240 - protein, 16 aa, synthetic construct
  REGION 1..16: note = Scaffold Protein
GGKLSKKKKGYNVNDE

SEQ ID NO: 241 - protein, 15 aa, synthetic construct
  REGION 1..15: note = Scaffold Protein
GGKLSKKKKGYNVND

SEQ ID NO: 242 - protein, 13 aa, synthetic construct
  REGION 1..13: note = Scaffold Protein
GGKLSKKKKGYNV

SEQ ID NO: 243 - protein, 12 aa, synthetic construct
  REGION 1..12: note = Scaffold Protein
GGKLSKKKKGYN

SEQ ID NO: 244 - protein, 11 aa, synthetic construct
  REGION 1..11: note = Scaffold Protein
GGKLSKKKKGY

SEQ ID NO: 245 - protein, 10 aa, synthetic construct
  REGION 1..10: note = Scaffold Protein
GGKLSKKKKG

SEQ ID NO: 246 - protein, 9 aa, synthetic construct
  REGION 1..9: note = Scaffold Protein
GGKLSKKKK

SEQ ID NO: 247 - protein, 29 aa, synthetic construct
  REGION 1..29: note = Scaffold Protein
GAKKSKKRFSFKKSFKLSGFSFKKNKKEA

SEQ ID NO: 248 - protein, 28 aa, synthetic construct
  REGION 1..28: note = Scaffold Protein
GAKKSKKRFSFKKSFKLSGFSFKKNKKE

SEQ ID NO: 249 - protein, 27 aa, synthetic construct
  REGION 1..27: note = Scaffold Protein
GAKKSKKRFSFKKSFKLSGFSFKKNKK

SEQ ID NO: 250 - protein, 26 aa, synthetic construct
  REGION 1..26: note = Scaffold Protein
GAKKSKKRFSFKKSFKLSGFSFKKNK

SEQ ID NO: 251 - protein, 25 aa, synthetic construct
  REGION 1..25: note = Scaffold Protein
GAKKSKKRFSFKKSFKLSGFSFKKN

SEQ ID NO: 252 - protein, 24 aa, synthetic construct
  REGION 1..24: note = Scaffold Protein
GAKKSKKRFSFKKSFKLSGFSFKK

SEQ ID NO: 253 - protein, 23 aa, synthetic construct
  REGION 1..23: note = Scaffold Protein
GAKKSKKRFSFKKSFKLSGFSFK

SEQ ID NO: 254 - protein, 22 aa, synthetic construct
  REGION 1..22: note = Scaffold Protein
GAKKSKKRFSFKKSFKLSGFSF

SEQ ID NO: 255 - protein, 21 aa, synthetic construct
  REGION 1..21: note = Scaffold Protein
GAKKSKKRFSFKKSFKLSGFS

SEQ ID NO: 256 - protein, 20 aa, synthetic construct
  REGION 1..20: note = Scaffold Protein
GAKKSKKRFSFKKSFKLSGF

SEQ ID NO: 257 - protein, 19 aa, synthetic construct
  REGION 1..19: note = Scaffold Protein
GAKKSKKRFSFKKSFKLSG

SEQ ID NO: 258 - protein, 18 aa, synthetic construct
  REGION 1..18: note = Scaffold Protein
GAKKSKKRFSFKKSFKLS

SEQ ID NO: 259 - protein, 17 aa, synthetic construct
  REGION 1..17: note = Scaffold Protein
GAKKSKKRFSFKKSFKL

SEQ ID NO: 260 - protein, 16 aa, synthetic construct
  REGION 1..16: note = Scaffold Protein
GAKKSKKRFSFKKSFK

SEQ ID NO: 261 - protein, 15 aa, synthetic construct
  REGION 1..15: note = Scaffold Protein
GAKKSKKRFSFKKSF

SEQ ID NO: 262 - protein, 13 aa, synthetic construct
  REGION 1..13: note = Scaffold Protein
GAKKSKKRFSFKK

SEQ ID NO: 263 - protein, 12 aa, synthetic construct
  REGION 1..12: note = Scaffold Protein
GAKKSKKRFSFK

SEQ ID NO: 264 - protein, 11 aa, synthetic construct
  REGION 1..11: note = Scaffold Protein
GAKKSKKRFSF

SEQ ID NO: 265 - protein, 10 aa, synthetic construct
  REGION 1..10: note = Scaffold Protein
GAKKSKKRFS

SEQ ID NO: 266 - protein, 9 aa, synthetic construct
  REGION 1..9: note = Scaffold Protein
GAKKSKKRF

SEQ ID NO: 267 - protein, 8 aa, synthetic construct
  REGION 1..8: note = Scaffold Protein
GAKKSKKR

SEQ ID NO: 268 - protein, 7 aa, synthetic construct
  REGION 1..7: note = Scaffold Protein
GAKKSKK

SEQ ID NO: 269 - protein, 29 aa, synthetic construct
  REGION 1..29: note = Scaffold Protein
GAKKAKKRFSFKKSFKLSGFSFKKNKKEA

SEQ ID NO: 270 - protein, 28 aa, synthetic construct
  REGION 1..28: note = Scaffold Protein
GAKKAKKRFSFKKSFKLSGFSFKKNKKE

SEQ ID NO: 271 - protein, 27 aa, synthetic construct
  REGION 1..27: note = Scaffold Protein
GAKKAKKRFSFKKSFKLSGFSFKKNKK

SEQ ID NO: 272 - protein, 26 aa, synthetic construct
  REGION 1..26: note = Scaffold Protein
GAKKAKKRFSFKKSFKLSGFSFKKNK

SEQ ID NO: 273 - protein, 25 aa, synthetic construct
  REGION 1..25: note = Scaffold Protein
GAKKAKKRFSFKKSFKLSGFSFKKN

SEQ ID NO: 274 - protein, 24 aa, synthetic construct
  REGION 1..24: note = Scaffold Protein
GAKKAKKRFSFKKSFKLSGFSFKK

SEQ ID NO: 275 - protein, 23 aa, synthetic construct
  REGION 1..23: note = Scaffold Protein
GAKKAKKRFSFKKSFKLSGFSFK

SEQ ID NO: 276 - protein, 22 aa, synthetic construct
  REGION 1..22: note = Scaffold Protein
GAKKAKKRFSFKKSFKLSGFSF

SEQ ID NO: 277 - protein, 21 aa, synthetic construct
  REGION 1..21: note = Scaffold Protein
GAKKAKKRFSFKKSFKLSGFS

SEQ ID NO: 278 - protein, 20 aa, synthetic construct
  REGION 1..20: note = Scaffold Protein
GAKKAKKRFSFKKSFKLSGF

SEQ ID NO: 279 - protein, 19 aa, synthetic construct
  REGION 1..19: note = Scaffold Protein
GAKKAKKRFSFKKSFKLSG

SEQ ID NO: 280 - protein, 18 aa, synthetic construct
  REGION 1..18: note = Scaffold Protein
GAKKAKKRFSFKKSFKLS

SEQ ID NO: 281 - protein, 17 aa, synthetic construct
  REGION 1..17: note = Scaffold Protein
GAKKAKKRFSFKKSFKL

SEQ ID NO: 282 - protein, 16 aa, synthetic construct
  REGION 1..16: note = Scaffold Protein
GAKKAKKRFSFKKSFK

SEQ ID NO: 283 - protein, 15 aa, synthetic construct
  REGION 1..15: note = Scaffold Protein
GAKKAKKRFSFKKSF

SEQ ID NO: 284 - protein, 14 aa, synthetic construct
  REGION 1..14: note = Scaffold Protein
GAKKAKKRFSFKKS

SEQ ID NO: 285 - protein, 13 aa, synthetic construct
  REGION 1..13: note = Scaffold Protein
GAKKAKKRFSFKK

SEQ ID NO: 286 - protein, 12 aa, synthetic construct
  REGION 1..12: note = Scaffold Protein
GAKKAKKRFSFK

SEQ ID NO: 287 - protein, 11 aa, synthetic construct
  REGION 1..11: note = Scaffold Protein
GAKKAKKRFSF

SEQ ID NO: 288 - protein, 10 aa, synthetic construct
  REGION 1..10: note = Scaffold Protein
GAKKAKKRFS

SEQ ID NO: 289 - protein, 9 aa, synthetic construct
  REGION 1..9: note = Scaffold Protein
GAKKAKKRF

SEQ ID NO: 290 - protein, 8 aa, synthetic construct
  REGION 1..8: note = Scaffold Protein
GAKKAKKR

SEQ ID NO: 291 - protein, 7 aa, synthetic construct
  REGION 1..7: note = Scaffold Protein
GAKKAKK

SEQ ID NO: 292 - protein, 28 aa, synthetic construct
  REGION 1..28: note = Scaffold Protein
GAQESKKKKKKRFSFKKSFKLSGFSFKK

SEQ ID NO: 293 - protein, 27 aa, synthetic construct
  REGION 1..27: note = Scaffold Protein
GAQESKKKKKKRFSFKKSFKLSGFSFK

SEQ ID NO: 294 - protein, 26 aa, synthetic construct
  REGION 1..26: note = Scaffold Protein
GAQESKKKKKKRFSFKKSFKLSGFSF

SEQ ID NO: 295 - protein, 25 aa, synthetic construct
  REGION 1..25: note = Scaffold Protein
GAQESKKKKKKRFSFKKSFKLSGFS

SEQ ID NO: 296 - protein, 24 aa, synthetic construct
  REGION 1..24: note = Scaffold Protein
GAQESKKKKKKRFSFKKSFKLSGF

SEQ ID NO: 297 - protein, 23 aa, synthetic construct
  REGION 1..23: note = Scaffold Protein
GAQESKKKKKKRFSFKKSFKLSG

SEQ ID NO: 298 - protein, 22 aa, synthetic construct
  REGION 1..22: note = Scaffold Protein
GAQESKKKKKKRFSFKKSFKLS

SEQ ID NO: 299 - protein, 21 aa, synthetic construct
  REGION 1..21: note = Scaffold Protein
GAQESKKKKKKRFSFKKSFKL

SEQ ID NO: 300 - protein, 20 aa, synthetic construct
  REGION 1..20: note = Scaffold Protein
GAQESKKKKKKRFSFKKSFK

SEQ ID NO: 301 - protein, 19 aa, synthetic construct
  REGION 1..19: note = Scaffold Protein
GAQESKKKKKKRFSFKKSF

SEQ ID NO: 302 - protein, 18 aa, synthetic construct
  REGION 1..18: note = Scaffold Protein
GAQESKKKKKKRFSFKKS

SEQ ID NO: 303 - protein, 17 aa, synthetic construct
  REGION 1..17: note = Scaffold Protein
GAQESKKKKKKRFSFKK

SEQ ID NO: 304 - protein, 16 aa, synthetic construct
  REGION 1..16: note = Scaffold Protein
GAQESKKKKKKRFSFK

SEQ ID NO: 305 - protein, 15 aa, synthetic construct
  REGION 1..15: note = Scaffold Protein
GAQESKKKKKKRFSF

SEQ ID NO: 306 - protein, 14 aa, synthetic construct
  REGION 1..14: note = Scaffold Protein
GAQESKKKKKKRFS

SEQ ID NO: 307 - protein, 13 aa, synthetic construct
  REGION 1..13: note = Scaffold Protein
GAQESKKKKKKRF

SEQ ID NO: 308 - protein, 12 aa, synthetic construct
  REGION 1..12: note = Scaffold Protein
GAQESKKKKKKR

SEQ ID NO: 309 - protein, 11 aa, synthetic construct
  REGION 1..11: note = Scaffold Protein
GAQESKKKKKK

SEQ ID NO: 310 - protein, 10 aa, synthetic construct
  REGION 1..10: note = Scaffold Protein
GAQESKKKKK

SEQ ID NO: 311 - protein, 9 aa, synthetic construct
  REGION 1..9: note = Scaffold Protein
GAQESKKKK

SEQ ID NO: 312 - protein, 8 aa, synthetic construct
  REGION 1..8: note = Scaffold Protein
GAQESKKK

SEQ ID NO: 313 - protein, 7 aa, synthetic construct
  REGION 1..7: note = Scaffold Protein
GAQESKK

SEQ ID NO: 314 - protein, 30 aa, synthetic construct
  REGION 1..30: note = Scaffold Protein
GSQSSKKKKKKFSFKKPFKLSGLSFKRNRK

SEQ ID NO: 315 - protein, 29 aa, synthetic construct
  REGION 1..29: note = Scaffold Protein
GSQSSKKKKKKFSFKKPFKLSGLSFKRNR

SEQ ID NO: 316 - protein, 28 aa, synthetic construct
  REGION 1..28: note = Scaffold Protein
GSQSSKKKKKKFSFKKPFKLSGLSFKRN

SEQ ID NO: 317 - protein, 27 aa, synthetic construct
  REGION 1..27: note = Scaffold Protein
GSQSSKKKKKKFSFKKPFKLSGLSFKR

SEQ ID NO: 318 - protein, 26 aa, synthetic construct
  REGION 1..26: note = Scaffold Protein
GSQSSKKKKKKFSFKKPFKLSGLSFK

SEQ ID NO: 319 - protein, 25 aa, synthetic construct
  REGION 1..25: note = Scaffold Protein
GSQSSKKKKKKFSFKKPFKLSGLSF

SEQ ID NO: 320 - protein, 24 aa, synthetic construct
  REGION 1..24: note = Scaffold Protein
GSQSSKKKKKKFSFKKPFKLSGLS

SEQ ID NO: 321 - protein, 23 aa, synthetic construct
  REGION 1..23: note = Scaffold Protein
GSQSSKKKKKKFSFKKPFKLSGL

SEQ ID NO: 322 - protein, 22 aa, synthetic construct
  REGION 1..22: note = Scaffold Protein
GSQSSKKKKKKFSFKKPFKLSG

SEQ ID NO: 323 - protein, 21 aa, synthetic construct
  REGION 1..21: note = Scaffold Protein
GSQSSKKKKKKFSFKKPFKLS

SEQ ID NO: 324 - protein, 20 aa, synthetic construct
  REGION 1..20: note = Scaffold Protein
GSQSSKKKKKKFSFKKPFKL

SEQ ID NO: 325 - protein, 19 aa, synthetic construct
  REGION 1..19: note = Scaffold Protein
GSQSSKKKKKKFSFKKPFK

SEQ ID NO: 326 - protein, 18 aa, synthetic construct
  REGION 1..18: note = Scaffold Protein
GSQSSKKKKKKFSFKKPF

SEQ ID NO: 327 - protein, 17 aa, synthetic construct
  REGION 1..17: note = Scaffold Protein
GSQSSKKKKKKFSFKKP

SEQ ID NO: 328 - protein, 16 aa, synthetic construct
  REGION 1..16: note = Scaffold Protein
GSQSSKKKKKKFSFKK

SEQ ID NO: 329 - protein, 15 aa, synthetic construct
  REGION 1..15: note = Scaffold Protein
GSQSSKKKKKKFSFK

SEQ ID NO: 330 - protein, 14 aa, synthetic construct
  REGION 1..14: note = Scaffold Protein
GSQSSKKKKKKFSF

SEQ ID NO: 331 - protein, 13 aa, synthetic construct
  REGION 1..13: note = Scaffold Protein
GSQSSKKKKKKFS

SEQ ID NO: 332 - protein, 12 aa, synthetic construct
  REGION 1..12: note = Scaffold Protein
GSQSSKKKKKKF

SEQ ID NO: 333 - protein, 11 aa, synthetic construct
  REGION 1..11: note = Scaffold Protein
GSQSSKKKKKK

SEQ ID NO: 334 - protein, 10 aa, synthetic construct
  REGION 1..10: note = Scaffold Protein
GSQSSKKKKK

SEQ ID NO: 335 - protein, 9 aa, synthetic construct
  REGION 1..9: note = Scaffold Protein
GSQSSKKKK

SEQ ID NO: 336 - protein, 8 aa, synthetic construct
  REGION 1..8: note = Scaffold Protein
GSQSSKKK

SEQ ID NO: 337 - protein, 7 aa, synthetic construct
  REGION 1..7: note = Scaffold Protein
GSQSSKK

SEQ ID NO: 338 - protein, 7 aa, synthetic construct
  REGION 1..7: note = fusion protein
GGKFSKK

SEQ ID NO: 339 - protein, 7 aa, synthetic construct
  REGION 1..7: note = fusion protein
GGKFAKK

SEQ ID NO: 340 - protein, 7 aa, synthetic construct
  REGION 1..7: note = fusion protein
GGKSSKK

SEQ ID NO: 341 - protein, 7 aa, synthetic construct
  REGION 1..7: note = fusion protein
GGKSAKK

SEQ ID NO: 342 - protein, 7 aa, synthetic construct
  REGION 1..7: note = fusion protein
GGKQAKK

SEQ ID NO: 343 - protein, 7 aa, synthetic construct
  REGION 1..7: note = fusion protein
GGQLSKK

SEQ ID NO: 344 - protein, 7 aa, synthetic construct
  REGION 1..7: note = fusion protein
GGQLAKK

SEQ ID NO: 345 - protein, 7 aa, synthetic construct
  REGION 1..7: note = fusion protein
GGQFSKK

SEQ ID NO: 346 - protein, 7 aa, synthetic construct
  REGION 1..7: note = fusion protein
GGQFAKK

SEQ ID NO: 347 - protein, 7 aa, synthetic construct
  REGION 1..7: note = fusion protein
GGQSSKK

SEQ ID NO: 348 - protein, 7 aa, synthetic construct
  REGION 1..7: note = fusion protein
GGQSAKK

SEQ ID NO: 349 - protein, 7 aa, synthetic construct
  REGION 1..7: note = fusion protein
GGQQSKK

SEQ ID NO: 350 - protein, 7 aa, synthetic construct
  REGION 1..7: note = fusion protein
GGQQAKK

SEQ ID NO: 351 - protein, 7 aa, synthetic construct
  REGION 1..7: note = fusion protein
GAKLAKK

SEQ ID NO: 352 - protein, 7 aa, synthetic construct
  REGION 1..7: note = fusion protein
GAKFSKK

SEQ ID NO: 353 - protein, 7 aa, synthetic construct
  REGION 1..7: note = fusion protein
GAKFAKK

SEQ ID NO: 354 - protein, 7 aa, synthetic construct
  REGION 1..7: note = fusion protein
GAKSSKK

SEQ ID NO: 355 - protein, 7 aa, synthetic construct
  REGION 1..7: note = fusion protein
GAKSAKK

SEQ ID NO: 356 - protein, 7 aa, synthetic construct
  REGION 1..7: note = fusion protein
GAKQSKK

SEQ ID NO: 357 - protein, 7 aa, synthetic construct
  REGION 1..7: note = fusion protein
GAKQAKK

SEQ ID NO: 358 - protein, 7 aa, synthetic construct
  REGION 1..7: note = fusion protein
GAQLSKK

SEQ ID NO: 359 - protein, 7 aa, synthetic construct
  REGION 1..7: note = fusion protein
GAQLAKK

SEQ ID NO: 360 - protein, 7 aa, synthetic construct
  REGION 1..7: note = fusion protein
GAQFSKK

SEQ ID NO: 361 - protein, 7 aa, synthetic construct
  REGION 1..7: note = fusion protein
GAQFAKK

SEQ ID NO: 362 - protein, 7 aa, synthetic construct
  REGION 1..7: note = fusion protein
GAQSSKK

SEQ ID NO: 363 - protein, 7 aa, synthetic construct
  REGION 1..7: note = fusion protein
GAQSAKK

SEQ ID NO: 364 - protein, 7 aa, synthetic construct
  REGION 1..7: note = fusion protein
GAQQSKK

SEQ ID NO: 365 - protein, 7 aa, synthetic construct
  REGION 1..7: note = fusion protein
GAQQAKK

SEQ ID NO: 366 - protein, 7 aa, synthetic construct
  REGION 1..7: note = fusion protein
GSKLSKK

SEQ ID NO: 367 - protein, 7 aa, synthetic construct
  REGION 1..7: note = fusion protein
GSKLAKK

SEQ ID NO: 368 - protein, 7 aa, synthetic construct
  REGION 1..7: note = fusion protein
GSKFSKK

SEQ ID NO: 369 - protein, 7 aa, synthetic construct
  REGION 1..7: note = fusion protein
GSKFAKK

SEQ ID NO: 370 - protein, 7 aa, synthetic construct
  REGION 1..7: note = fusion protein
GSKSSKK

SEQ ID NO: 371 - protein, 7 aa, synthetic construct
  REGION 1..7: note = fusion protein
GSKSAKK

SEQ ID NO: 372 - protein, 7 aa, synthetic construct
  REGION 1..7: note = fusion protein
GSKQSKK

SEQ ID NO: 373 - protein, 7 aa, synthetic construct
  REGION 1..7: note = fusion protein
GSKQAKK

SEQ ID NO: 374 - protein, 7 aa, synthetic construct
  REGION 1..7: note = fusion protein
GSQLSKK

SEQ ID NO: 375 - protein, 7 aa, synthetic construct
  REGION 1..7: note = fusion protein
GSQLAKK

SEQ ID NO: 376 - protein, 7 aa, synthetic construct
  REGION 1..7: note = fusion protein
GSQFSKK

SEQ ID NO: 377 - protein, 7 aa, synthetic construct
  REGION 1..7: note = fusion protein
GSQFAKK

SEQ ID NO: 378 - protein, 7 aa, synthetic construct
  REGION 1..7: note = fusion protein
GSQSAKK

SEQ ID NO: 379 - protein, 7 aa, synthetic construct
  REGION 1..7: note = fusion protein
GSQQSKK

SEQ ID NO: 380 - protein, 7 aa, synthetic construct
  REGION 1..7: note = fusion protein
GSQQAKK

SEQ ID NO: 381 - protein, 6 aa, synthetic construct
  REGION 1..6: note = fusion protein
GGKFSK

SEQ ID NO: 382 - protein, 6 aa, synthetic construct
  REGION 1..6: note = fusion protein
GGKFAK

SEQ ID NO: 383 - protein, 6 aa, synthetic construct
  REGION 1..6: note = fusion protein
GGKSSK

SEQ ID NO: 384 - protein, 6 aa, synthetic construct
  REGION 1..6: note = fusion protein
GGKSAK

SEQ ID NO: 385 - protein, 6 aa, synthetic construct
  REGION 1..6: note = fusion protein
GGKQAK

SEQ ID NO: 386 - protein, 6 aa, synthetic construct
  REGION 1..6: note = fusion protein
GGQLSK

SEQ ID NO: 387 - protein, 6 aa, synthetic construct
  REGION 1..6: note = fusion protein
GGQLAK

SEQ ID NO: 388 - protein, 6 aa, synthetic construct
  REGION 1..6: note = fusion protein
GGQFSK

SEQ ID NO: 389 - protein, 6 aa, synthetic construct
  REGION 1..6: note = fusion protein
GGQFAK

SEQ ID NO: 390 - protein, 6 aa, synthetic construct
  REGION 1..6: note = fusion protein
GGQSSK

SEQ ID NO: 391 - protein, 6 aa, synthetic construct
  REGION 1..6: note = fusion protein
GGQSAK

SEQ ID NO: 392 - protein, 6 aa, synthetic construct
  REGION 1..6: note = fusion protein
GGQQSK

SEQ ID NO: 393 - protein, 6 aa, synthetic construct
  REGION 1..6: note = fusion protein
GGQQAK

SEQ ID NO: 394 - protein, 6 aa, synthetic construct
  REGION 1..6: note = fusion protein
GAKLAK

SEQ ID NO: 395 - protein, 6 aa, synthetic construct
  REGION 1..6: note = fusion protein
GAKFSK

SEQ ID NO: 396 - protein, 6 aa, synthetic construct
  REGION 1..6: note = fusion protein
GAKFAK

SEQ ID NO: 397 - protein, 6 aa, synthetic construct
  REGION 1..6: note = fusion protein
GAKSSK

SEQ ID NO: 398 - protein, 6 aa, synthetic construct
  REGION 1..6: note = fusion protein
GAKSAK

SEQ ID NO: 399 - protein, 6 aa, synthetic construct
  REGION 1..6: note = fusion protein
GAKQSK

SEQ ID NO: 400 - protein, 6 aa, synthetic construct
  REGION 1..6: note = fusion protein
GAKQAK

SEQ ID NO: 401 - protein, 6 aa, synthetic construct
  REGION 1..6: note = fusion protein
GAQLSK

SEQ ID NO: 402 - protein, 6 aa, synthetic construct
  REGION 1..6: note = fusion protein
GAQLAK

SEQ ID NO: 403 - protein, 6 aa, synthetic construct
  REGION 1..6: note = fusion protein
GAQFSK

SEQ ID NO: 404 - protein, 6 aa, synthetic construct
  REGION 1..6: note = fusion protein
GAQFAK

SEQ ID NO: 405 - protein, 6 aa, synthetic construct
  REGION 1..6: note = fusion protein
GAQSSK

SEQ ID NO: 406 - protein, 6 aa, synthetic construct
  REGION 1..6: note = fusion protein
GAQSAK

SEQ ID NO: 407 - protein, 6 aa, synthetic construct
  REGION 1..6: note = fusion protein
GAQQSK

SEQ ID NO: 408 - protein, 6 aa, synthetic construct
  REGION 1..6: note = fusion protein
GAQQAK

SEQ ID NO: 409 - protein, 6 aa, synthetic construct
  REGION 1..6: note = fusion protein
GSKLSK

SEQ ID NO: 410 - protein, 6 aa, synthetic construct
  REGION 1..6: note = fusion protein
GSKLAK

SEQ ID NO: 411 - protein, 6 aa, synthetic construct
  REGION 1..6: note = fusion protein
GSKFSK

SEQ ID NO: 412 - protein, 6 aa, synthetic construct
  REGION 1..6: note = fusion protein
GSKFAK

SEQ ID NO: 413 - protein, 6 aa, synthetic construct
  REGION 1..6: note = fusion protein
GSKSSK

SEQ ID NO: 414 - protein, 6 aa, synthetic construct
  REGION 1..6: note = fusion protein
GSKSAK

SEQ ID NO: 415 - protein, 6 aa, synthetic construct
  REGION 1..6: note = fusion protein
GSKQSK

SEQ ID NO: 416 - protein, 6 aa, synthetic construct
  REGION 1..6: note = fusion protein
GSKQAK

SEQ ID NO: 417 - protein, 6 aa, synthetic construct
  REGION 1..6: note = fusion protein
GSQLSK

SEQ ID NO: 418 - protein, 6 aa, synthetic construct
  REGION 1..6: note = fusion protein
GSQLAK

SEQ ID NO: 419 - protein, 6 aa, synthetic construct
  REGION 1..6: note = fusion protein
GSQFSK

SEQ ID NO: 420 - protein, 6 aa, synthetic construct
  REGION 1..6: note = fusion protein
GSQFAK

SEQ ID NO: 421 - protein, 6 aa, synthetic construct
  REGION 1..6: note = fusion protein
GSQSSK

SEQ ID NO: 422 - protein, 6 aa, synthetic construct
  REGION 1..6: note = fusion protein
GSQSAK

SEQ ID NO: 423 - protein, 6 aa, synthetic construct
  REGION 1..6: note = fusion protein
GSQQSK

SEQ ID NO: 424 - protein, 6 aa, synthetic construct
  REGION 1..6: note = fusion protein
GSQQAK

SEQ ID NO: 425 - protein, 8 aa, synthetic construct
  REGION 1..8: note = Fusion Protein
  SITE 2: note = misc_feature - Xaa can be any naturally occurring amino acid
GXKLSKKK